European Patent Application EP 4 455 300 A1, published October 30, 2024. Title: Method For Preparing a Microsphere Chip and Related Application. Applicant: BEIJING BIOMARKER TECHNOLOGY CO.,LTD. The sequence listing filed with the application follows.

SEQUENCE LISTING (49 sequences)

SEQ ID NO: 1 - DNA, 59 bp, synthetic construct
  source 1..59: mol_type = other DNA
ctacacgacgctcttccgatctctgcgctcacaatactagtcatcgcagagtactacgt

SEQ ID NO: 2 - DNA, 59 bp, synthetic construct
  source 1..59: mol_type = other DNA
ctacacgacgctcttccgatctcgtaagggcatggttgagtcatcgcagagtactacgt

SEQ ID NO: 3 - DNA, 59 bp, synthetic construct
  source 1..59: mol_type = other DNA
ctacacgacgctcttccgatctctgtcaagaacgttgacgtcatcgcagagtactacgt

SEQ ID NO: 4 - DNA, 59 bp, synthetic construct
  source 1..59: mol_type = other DNA
ctacacgacgctcttccgatctcgtcagcttactttgctgtcatcgcagagtactacgt

SEQ ID NO: 5 - DNA, 59 bp, synthetic construct
  source 1..59: mol_type = other DNA
ctacacgacgctcttccgatctacattgcaaggtgcacggtcatcgcagagtactacgt

SEQ ID NO: 6 - DNA, 59 bp, synthetic construct
  source 1..59: mol_type = other DNA
caactcactgtagtgagtcggattgagagctcctgttcgacgtagtactctgcgatgac

SEQ ID NO: 7 - DNA, 59 bp, synthetic construct
  source 1..59: mol_type = other DNA
caactcactgtagtgagtcgttgtgcggaacgtgaccatacgtagtactctgcgatgac

SEQ ID NO: 8 - DNA, 59 bp, synthetic construct
  source 1..59: mol_type = other DNA
caactcactgtagtgagtcgggaaagattctatccgtcgacgtagtactctgcgatgac

SEQ ID NO: 9 - DNA, 59 bp, synthetic construct
  source 1..59: mol_type = other DNA
caactcactgtagtgagtcgactcgttgagctaatcccgacgtagtactctgcgatgac

SEQ ID NO: 10 - DNA, 59 bp, synthetic construct
  source 1..59: mol_type = other DNA
caactcactgtagtgagtcgcccgggtcctaactattgcacgtagtactctgcgatgac

SEQ ID NO: 11 - DNA, 59 bp, synthetic construct
  source 1..59: mol_type = other DNA
ccagacgatcgtgtcactgacaatacgcatctcacagaccaactcactgtagtgagtcg

SEQ ID NO: 12 - DNA, 59 bp, synthetic construct
  source 1..59: mol_type = other DNA
ccagacgatcgtgtcactgatgtatacgtccgctgtcaacaactcactgtagtgagtcg

SEQ ID NO: 13 - DNA, 59 bp, synthetic construct
  source 1..59: mol_type = other DNA
ccagacgatcgtgtcactgaatgaggatacatgtcgagccaactcactgtagtgagtcg

SEQ ID NO: 14 - DNA, 59 bp, synthetic construct
  source 1..59: mol_type = other DNA
ccagacgatcgtgtcactgagcctacttaaccgccagatcaactcactgtagtgagtcg

SEQ ID NO: 15 - DNA, 59 bp, synthetic construct
  source 1..59: mol_type = other DNA
ccagacgatcgtgtcactgaaagccagctcagctacttccaactcactgtagtgagtcg

SEQ ID NO: 16 - DNA, 72 bp, synthetic construct
  source 1..72: mol_type = other DNA
  misc_feature 1: note = n is a, t, c or g
  misc_feature 2: note = b is g, t or c.
  misc_feature 33..52: note = n is a,t, g or c.
nbaaaaaaaaaaaaaaaaaaaaaaaaaaaaaannnnnnnnnnnnnnnnnnnnccagacgatcgtgtcactga

SEQ ID NO: 17 - DNA, 40 bp, synthetic construct
  source 1..40: mol_type = other DNA
ctacacgacgctcttccgatctctgcgctcacaatactag

SEQ ID NO: 18 - DNA, 41 bp, synthetic construct
  source 1..41: mol_type = other DNA
ctacacgacgctcttccgatctcgtaagggcatggttgagt

SEQ ID NO: 19 - DNA, 49 bp, synthetic construct
  source 1..49: mol_type = other DNA
ctacacgacgctcttccgatctctgtcaagaacgttgacgtcatcgcag

SEQ ID NO: 20 - DNA, 19 bp, synthetic construct
  source 1..19: mol_type = other DNA
cgggattagctcaacgagt

SEQ ID NO: 21 - DNA, 40 bp, synthetic construct
  source 1..40: mol_type = other DNA
gactcgttgagctaatcccgacgtagtactctgcgatgac

SEQ ID NO: 22 - DNA, 41 bp, synthetic construct
  source 1..41: mol_type = other DNA
cgactcgttgagctaatcccgacgtagtactctgcgatgac

SEQ ID NO: 23 - DNA, 49 bp, synthetic construct
  source 1..49: mol_type = other DNA
tagtgagtcgactcgttgagctaatcccgacgtagtactctgcgatgac

SEQ ID NO: 24 - DNA, 82 bp, synthetic construct
  source 1..82: mol_type = other DNA
  misc_feature 81: note = v is a, g or c.
  misc_feature 49..50: note = n is a, t, g or c.
  misc_feature 82: note = n is a, t, c or g.
cgactcactacagtgagttggctcgacatgtatcctcatnnnnnnnnnnnntttttttttttttttttttttttttttttvn

SEQ ID NO: 25 - DNA, 15 bp, synthetic construct
  source 1..15: mol_type = other DNA
  misc_feature 1: note = cy5 modification
aaaaaaaaaaaaaaa

SEQ ID NO: 26 - DNA, 44 bp, synthetic construct
  source 1..44: mol_type = other DNA
ctacacgacgctcttccgatcttttagctctcctatggctacgt

SEQ ID NO: 27 - DNA, 44 bp, synthetic construct
  source 1..44: mol_type = other DNA
ctacacgacgctcttccgatctcgagctcaaggatatcgtacgt

SEQ ID NO: 28 - DNA, 44 bp, synthetic construct
  source 1..44: mol_type = other DNA
ctacacgacgctcttccgatctggcgtaaggaccttacgtacgt

SEQ ID NO: 29 - DNA, 44 bp, synthetic construct
  source 1..44: mol_type = other DNA
ctacacgacgctcttccgatcttcgcttacaaatctggttacgt

SEQ ID NO: 30 - DNA, 19 bp, synthetic construct
  source 1..19: mol_type = other DNA
ttcttcacagccagcctag

SEQ ID NO: 31 - DNA, 19 bp, synthetic construct
  source 1..19: mol_type = other DNA
tataggtgacctgcagtaa

SEQ ID NO: 32 - DNA, 19 bp, synthetic construct
  source 1..19: mol_type = other DNA
ccatatacgtgctaccaaa

SEQ ID NO: 33 - DNA, 19 bp, synthetic construct
  source 1..19: mol_type = other DNA
cacatacttgcgggttgag

SEQ ID NO: 34 - DNA, 59 bp, synthetic construct
  source 1..59: mol_type = other DNA
  misc_feature 26..37: note = n is a, t, c or g.
  misc_feature 58: note = v is a, g or c.
  misc_feature 59: note = n is a, t, c or g.
cgactcttgacgtcgaagtccttcgnnnnnnnnnnnnttttttttttttttttttttvn

SEQ ID NO: 35 - DNA, 59 bp, synthetic construct
  source 1..59: mol_type = other DNA
  misc_feature 26..37: note = n is a, t, c or g.
  misc_feature 59: note = n is a, t, c or g.
  misc_feature 58: note = v is a, g or c.
cgactcgaggtacatgctacccgacnnnnnnnnnnnnttttttttttttttttttttvn

SEQ ID NO: 36 - DNA, 59 bp, synthetic construct
  source 1..59: mol_type = other DNA
  misc_feature 26..37: note = n is a, t, c or g.
  misc_feature 59: note = n is a, t, c or g.
  misc_feature 58: note = v is a, g or c.
cgactcatgcatgtgtcagtgtggcnnnnnnnnnnnnttttttttttttttttttttvn

SEQ ID NO: 37 - DNA, 59 bp, synthetic construct
  source 1..59: mol_type = other DNA
  misc_feature 26..39: note = n is a, t, c or g.
  misc_feature 59: note = n is a, t, c or g.
  misc_feature 58: note = v is a, g or c.
cgactccattatgaggtaaccctagnnnnnnnnnnnnttttttttttttttttttttvn

SEQ ID NO: 38 - DNA, 17 bp, synthetic construct
  source 1..17: mol_type = other DNA
gccataggagagctaaa

SEQ ID NO: 39 - DNA, 17 bp, synthetic construct
  source 1..17: mol_type = other DNA
cgatatccttgagctcg

SEQ ID NO: 40 - DNA, 17 bp, synthetic construct
  source 1..17: mol_type = other DNA
cgtaaggtccttacgcc

SEQ ID NO: 41 - DNA, 17 bp, synthetic construct
  source 1..17: mol_type = other DNA
accagatttgtaagcga

SEQ ID NO: 42 - DNA, 19 bp, synthetic construct
  source 1..19: mol_type = other DNA
ctaggctggctgtgaagaa

SEQ ID NO: 43 - DNA, 19 bp, synthetic construct
  source 1..19: mol_type = other DNA
ttactgcaggtcacctata

SEQ ID NO: 44 - DNA, 19 bp, synthetic construct
  source 1..19: mol_type = other DNA
tttggtagcacgtatatgg

SEQ ID NO: 45 - DNA, 19 bp, synthetic construct
  source 1..19: mol_type = other DNA
ctcaacccgcaagtatgtg

SEQ ID NO: 46 - DNA, 19 bp, synthetic construct
  source 1..19: mol_type = other DNA
cgaaggacttcgacgtcaa

SEQ ID NO: 47 - DNA, 19 bp, synthetic construct
  source 1..19: mol_type = other DNA
gtcgggtagcatgtacctc

SEQ ID NO: 48 - DNA, 19 bp, synthetic construct
  source 1..19: mol_type = other DNA
gccacactgacacatgcat

SEQ ID NO: 49 - DNA, 19 bp, synthetic construct
  source 1..19: mol_type = other DNA
ctagggttacctcataatg